European Patent Specification EP 3 844 287 B1, published May 22, 2024. Title: COMPOSITIONS AND METHODS FOR ENHANCING DONOR OLIGONUCLEOTIDE-BASED GENE EDITING. Applicant: YALE UNIVERSITY QUIJANO, ELIAS TURCHICK, AUDREY GLAZER, PETER. The sequence listing filed with the application follows.

SEQUENCE LISTING (53 sequences)

SEQ ID NO: 1 - protein, 116 aa, Artificial Sequence
  synthetic polypeptide
EVQLVESGGGLVKPGGSRKLSCAASGFTFSDYGMHWVRQAPEKGLEWVAYISSGSSTIYYADTVKGRFTISRDNAKNTLFLQMTSLRSEDTAMYYCARRGLLLDYWGQGTTLTVSS

SEQ ID NO: 2 - protein, 116 aa, Artificial Sequence
  synthetic polypeptide
EVQLVESGGGLVKPGGSRKLSCAASGFTFSNYGMHWVRQAPEKGLEWVAYISSGSSTIYYADTVKGRFTISRDNAKNTLFLQMTSLRSEDTAMYYCARRGLLLDYWGQGTTLTVSS

SEQ ID NO: 3 - protein, 116 aa, Artificial Sequence
  synthetic polypeptide
EVQLVQSGGGLIQPGGSLRLSCAASGFTFSNYGMHWVRQAPGKGLEWVSYISSGSSTIYYADSVKGRFTISRDNSKNTLYLQMNSLRAEDTAVYYCARRGLLLDYWGQGTTVTVSS

SEQ ID NO: 4 - protein, 116 aa, Artificial Sequence
  synthetic polypeptide
EVQLVESGGGLIQPGGSLRLSCAASGFTFSNYGMHWVRQAPGKGLEWVSYISSGSSTIYYADSVKGRFTISRDNSKNTLYLQMTSLRAEDTAVYYCARRGLLLDYWGQGTTLTVSS

SEQ ID NO: 5 - protein, 116 aa, Artificial Sequence
  synthetic polypeptide
EVQLQESGGGVVQPGGSLRLSCAASGFTFSNYGMHWIRQAPGKGLEWVSYISSGSSTIYYADSVKGRFTISRDNSKNTLYLQMNSLRSEDTAVYYCARRGLLLDYWGQGTLVTVSS

SEQ ID NO: 6 - protein, 116 aa, Artificial Sequence
  synthetic polypeptide
EVQLVESGGGLVQPGGSLRLSCSASGFTFSNYGMHWVRQAPGKGLEYVSYISSGSSTIYYADTVKGRFTISRDNSKNTLYLQMSSLRAEDTAVYYCVKRGLLLDYWGQGTLVTVSS

SEQ ID NO: 7 - protein, 111 aa, Artificial Sequence
  synthetic polypeptide
DIVLTQSPASLAVSLGQRATISCRASKSVSTSSYSYMHWYQQKPGQPPKLLIKYASYLESGVPARFSGSGSGTDFTLNIHPVEEEDAATYYCQHSREFPWTFGGGTKLEIK

SEQ ID NO: 8 - protein, 111 aa, Artificial Sequence
  synthetic polypeptide
DIVLTQSPASLAVSLGQRATISCRASKSVSTSSYSYMHWYQQKPGQPPKLLIKYASYLESGVPARFSGSGSGTDFHLNIHPVEEEDAATYYCQHSREFPWTFGGGTKLELK

SEQ ID NO: 9 - protein, 111 aa, Artificial Sequence
  synthetic polypeptide
DIQMTQSPSSLSASVGDRVTITCRASKSVSTSSYSYLAWYQQKPEKAPKLLIKYASYLQSGVPSRFSGSGSGTDFTLTISSLQPEDFATYYCQHSREFPWTFGAGTKLELK

SEQ ID NO: 10 - protein, 111 aa, Artificial Sequence
  synthetic polypeptide
DIQMTQSPSSLSASVGDRVTISCRASKSVSTSSYSYMHWYQQKPEKAPKLLIKYASYLQSGVPSRFSGSGSGTDFTLTISSLQPEDVATYYCQHSREFPWTFGAGTKLELK

SEQ ID NO: 11 - protein, 111 aa, Artificial Sequence
  synthetic polypeptide
DIVLTQSPASLAVSPGQRATITCRASKSVSTSSYSYMHWYQQKPGQPPKLLIYYASYLESGVPARFSGSGSGTDFTLTINPVEANDTANYYCQHSREFPWTFGQGTKVEIK

SEQ ID NO: 12 - protein, 465 aa, Artificial Sequence
  synthetic polypeptide
MGWSCIILFLVATATGVHSEVQLVESGGGLVKPGGSRKLSCAASGFTFSDYGMHWVRQAPEKGLEWVAYISSGSSTIYYADTVKGRFTISRDNAKNTLFLQMTSLRSEDTAMYYCARRGLLLDYWGQGTTLTVSAASTKGPSVFPLAPSSKSTSGGTAALGCLVKDYFPEPVTVSWNSGALTSGVHTFPAVLQSSGLYSLSSVVTVPSSSLGTQTYICNVNHKPSNTKVDKKVEPKSCDKTHTCPPCPAPELLGGPSVFLFPPKPKDTLMISRTPEVTCVVVDVSHEDPEVKFNWYVDGVEVHNAKTKPREEQYNSTYRVVSVLTVLHQDWLNGKEYKCKVSNKALPAPIEKTISKAKGQPREPQVYTLPPSRDELTKNQVSLTCLVKGFYPSDIAVEWESNGQPENNYKTTPPVLDSDGSFFLYSKLTVDKSRWQQGNVFSCSVMHEALHNHYTQKSLSLSPGK

SEQ ID NO: 13 - protein, 465 aa, Artificial Sequence
  synthetic polypeptide
MGWSCIILFLVATATGVHSEVQLVESGGGLVKPGGSRKLSCAASGFTFSNYGMHWVRQAPEKGLEWVAYISSGSSTIYYADTVKGRFTISRDNAKNTLFLQMTSLRSEDTAMYYCARRGLLLDYWGQGTTLTVSAASTKGPSVFPLAPSSKSTSGGTAALGCLVKDYFPEPVTVSWNSGALTSGVHTFPAVLQSSGLYSLSSVVTVPSSSLGTQTYICNVNHKPSNTKVDKKVEPKSCDKTHTCPPCPAPELLGGPSVFLFPPKPKDTLMISRTPEVTCVVVDVSHEDPEVKFNWYVDGVEVHNAKTKPREEQYNSTYRVVSVLTVLHQDWLNGKEYKCKVSNKALPAPIEKTISKAKGQPREPQVYTLPPSRDELTKNQVSLTCLVKGFYPSDIAVEWESNGQPENNYKTTPPVLDSDGSFFLYSKLTVDKSRWQQGNVFSCSVMHEALHNHYTQKSLSLSPGK

SEQ ID NO: 14 - protein, 237 aa, Artificial Sequence
  synthetic polypeptide
MGWSCIILFLVATATGVHSDIVLTQSPASLAVSLGQRATISCRASKSVSTSSYSYMHWYQQKPGQPPKLLIKYASYLESGVPARFSGSGSGTDFTLNIHPVEEEDAATYYCQHSREFPWTFGGGTKLEIKRTVAAPSVFIFPPSDEQLKSGTASVVCLLNNFYPREAKVQWKVDNALQSGNSQESVTEQDSKDSTYSLSSTLTLSKADYEKHKVYACEVTHQGLSSPVTKSFNRGEC

SEQ ID NO: 15 - protein, 5 aa, Artificial Sequence
  synthetic polypeptide
DYGMH

SEQ ID NO: 16 - protein, 5 aa, Artificial Sequence
  synthetic polypeptide
NYGMH

SEQ ID NO: 17 - protein, 17 aa, Artificial Sequence
  synthetic polypeptide
YISSGSSTIYYADTVKG

SEQ ID NO: 18 - protein, 7 aa, Artificial Sequence
  synthetic polypeptide
RGLLLDY

SEQ ID NO: 19 - protein, 17 aa, Artificial Sequence
  synthetic polypeptide
YISSGSSTIYYADSVKG

SEQ ID NO: 20 - protein, 8 aa, Artificial Sequence
  synthetic polypeptide
GFTFSDYG

SEQ ID NO: 21 - protein, 8 aa, Artificial Sequence
  synthetic polypeptide
GFTFSNYG

SEQ ID NO: 22 - protein, 8 aa, Artificial Sequence
  synthetic polypeptide
ISSGSSTI

SEQ ID NO: 23 - protein, 9 aa, Artificial Sequence
  synthetic polypeptide
ARRGLLLDY

SEQ ID NO: 24 - protein, 15 aa, Artificial Sequence
  synthetic polypeptide
RASKSVSTSSYSYMH

SEQ ID NO: 25 - protein, 7 aa, Artificial Sequence
  synthetic polypeptide
YASYLES

SEQ ID NO: 26 - protein, 9 aa, Artificial Sequence
  synthetic polypeptide
QHSREFPWT

SEQ ID NO: 27 - protein, 15 aa, Artificial Sequence
  synthetic polypeptide
RASKSVSTSSYSYLA

SEQ ID NO: 28 - protein, 7 aa, Artificial Sequence
  synthetic polypeptide
YASYLQS

SEQ ID NO: 29 - protein, 10 aa, Artificial Sequence
  synthetic polypeptide
KSVSTSSYSY

SEQ ID NO: 30 - protein, 3 aa, Artificial Sequence
  synthetic polypeptide
YAS

SEQ ID NO: 31 - protein, 7 aa, Artificial Sequence
  synthetic polypeptide
GQSSRSS

SEQ ID NO: 32 - protein, 18 aa, Artificial Sequence
  synthetic polypeptide
GQSSRSSSGGGSSGGGGS

SEQ ID NO: 33 - protein, 4 aa, Artificial Sequence
  synthetic polypeptide
GSGS

SEQ ID NO: 34 - protein, 4 aa, Artificial Sequence
  synthetic polypeptide
GGGS

SEQ ID NO: 35 - protein, 10 aa, Artificial Sequence
  synthetic polypeptide
GGGGSGGGGS

SEQ ID NO: 36 - protein, 20 aa, Artificial Sequence
  synthetic polypeptide
GGGGSGGGGSGGGGSGGGGS

SEQ ID NO: 37 - protein, 15 aa, Artificial Sequence
  synthetic polypeptide
GGGGSGGGGSGGGGS

SEQ ID NO: 38 - protein, 274 aa, Artificial Sequence
  synthetic polypeptide
AGIHDIVLTQSPASLAVSLGQRATISCRASKSVSTSSYSYMHWYQQKPGQPPKLLIKYASYLESGVPARFSGSGSGTDFTLNIHPVEEEDAATYYCQHSREFPWTFGGGTKLEIKRADAAPGGGGSGGGGSGGGGSEVQLVESGGGLVKPGGSRKLSCAASGFTFSNYGMHWVRQAPEKGLEWVAYISSGSSTIYYADTVKGRFTISRDNAKNTLFLQMTSLRSEDTAMYYCARRGLLLDYWGQGTTLTVSSLEQKLISEEDLNSAVDHHHHHH

SEQ ID NO: 39 - protein, 541 aa, Artificial Sequence
  synthetic polypeptide
AGIHDIVLTQSPASLAVSLGQRATISCRASKSVSTSSYSYMHWYQQKPGQPPKLLIKYASYLESGVPARFSGSGSGTDFTLNIHPVEEEDAATYYCQHSREFPWTFGGGTKLEIKRADAAPGGGGSGGGGSGGGGSEVQLVESGGGLVKPGGSRKLSCAASGFTFSNYGMHWVRQAPEKGLEWVAYISSGSSTIYYADTVKGRFTISRDNAKNTLFLQMTSLRSEDTAMYYCARRGLLLDYWGQGTTLTVSSASTKGPSVFPLAPLESSGSDIVLTQSPASLAVSLGQRATISCRASKSVSTSSYSYMHWYQQKPGQPPKLLIKYASYLESGVPARFSGSGSGTDFTLNIHPVEEEDAATYYCQHSREFPWTFGGGTKLEIKRADAAPGGGGSGGGGSGGGGSEVQLVESGGGLVKPGGSRKLSCAASGFTFSNYGMHWVRQAPEKGLEWVAYISSGSSTIYYADTVKGRFTISRDNAKNTLFLQMTSLRSEDTAMYYCARRGLLLDYWGQGTTLTVSSLEQKLISEEDLNSAVDHHHHHH

SEQ ID NO: 40 - protein, 808 aa, Artificial Sequence
  synthetic polypeptide
AGIHDIVLTQSPASLAVSLGQRATISCRASKSVSTSSYSYMHWYQQKPGQPPKLLIKYASYLESGVPARFSGSGSGTDFTLNIHPVEEEDAATYYCQHSREFPWTFGGGTKLEIKRADAAPGGGGSGGGGSGGGGSEVQLVESGGGLVKPGGSRKLSCAASGFTFSNYGMHWVRQAPEKGLEWVAYISSGSSTIYYADTVKGRFTISRDNAKNTLFLQMTSLRSEDTAMYYCARRGLLLDYWGQGTTLTVSSASTKGPSVFPLAPLESSGSDIVLTQSPASLAVSLGQRATISCRASKSVSTSSYSYMHWYQQKPGQPPKLLIKYASYLESGVPARFSGSGSGTDFTLNIHPVEEEDAATYYCQHSREFPWTFGGGTKLEIKRADAAPGGGGSGGGGSGGGGSEVQLVESGGGLVKPGGSRKLSCAASGFTFSNYGMHWVRQAPEKGLEWVAYISSGSSTIYYADTVKGRFTISRDNAKNTLFLQMTSLRSEDTAMYYCARRGLLLDYWGQGTTLTVSSASTKGPSVFPLAPLESSGSDIVLTQSPASLAVSLGQRATISCRASKSVSTSSYSYMHWYQQKPGQPPKLLIKYASYLESGVPARFSGSGSGTDFTLNIHPVEEEDAATYYCQHSREFPWTFGGGTKLEIKRADAAPGGGGSGGGGSGGGGSEVQLVESGGGLVKPGGSRKLSCAASGFTFSNYGMHWVRQAPEKGLEWVAYISSGSSTIYYADTVKGRFTISRDNAKNTLFLQMTSLRSEDTAMYYCARRGLLLDYWGQGTTLTVSSLEQKLISEEDLNSAVDHHHHHH

SEQ ID NO: 41 - protein, 242 aa, Artificial Sequence
  synthetic polypeptide
DIVLTQSPASLAVSPGQRATITCRASKSVSTSSYSYMHWYQQKPGQPPKLLIYYASYLESGVPARFSGSGSGTDFTLTINPVEANDTANYYCQHSREFPWTFGQGTKVEIKGGGGSGGGGSGGGGSEVQLVESGGGLVQPGGSLRLSCSASGFTFSNYGMHWVRQAPGKGLEYVSYISSGSSTIYYADTVKGRFTISRDNSKNTLYLQMSSLRAEDTAVYYCVKRGLLLDYWGQGTLVTVSS

SEQ ID NO: 42 - DNA, 6060 bp, Artificial Sequence
  synthetic polynucleotide
aaagctcttgctttgacaattttggtctttcagaatactataaatataacctatattataatttcataaagtctgtgcattttctttgacccaggatatttgcaaaagacatattcaaacttccgcagaacactttatttcacatatacatgcctcttatatcagggatgtgaaacagggtcttgaaaactgtctaaatctaaaacaatgctaatgcaggtttaaatttaataaaataaaatccaaaatctaacagccaagtcaaatctgtatgttttaacatttaaaatattttaaagacgtcttttcccaggattcaacatgtgaaatcttttctcagggatacacgtgtgcctagatcctcattgctttagttttttacagaggaatgaatataaaaagaaaatacttaaattttatccctcttacctctataatcatacataggcataattttttaacctaggctccagatagccatagaagaaccaaacactttctgcgtgtgtgagaataatcagagtgagattttttcacaagtacctgatgagggttgagacaggtagaaaaagtgagagatctctatttatttagcaataatagagaaagcatttaagagaataaagcaatggaaataagaaatttgtaaatttccttctgataactagaaatagaggatccagtttcttttggttaacctaaattttatttcattttattgttttattttattttattttattttattttgtgtaatcgtagtttcagagtgttagagctgaaaggaagaagtaggagaaacatgcaaagtaaaagtataacactttccttactaaaccgactgggtttccaggtaggggcaggattcaggatgactgacagggcccttagggaacactgagaccctacgctgacctcataaatgcttgctacctttgctgttttaattacatcttttaatagcaggaagcagaactctgcacttcaaaagtttttcctcacctgaggagttaatttagtacaaggggaaaaagtacagggggatgggagaaaggcgatcacgttgggaagctatagagaaagaagagtaaattttagtaaaggaggtttaaacaaacaaaatataaagagaaataggaacttgaatcaaggaaatgattttaaaacgcagtattcttagtggactagaggaaaaaaataatctgagccaagtagaagaccttttcccctcctacccctactttctaagtcacagaggctttttgttcccccagacactcttgcagattagtccaggcagaaacagttagatgtccccagttaacctcctatttgacaccactgattaccccattgatagtcacactttgggttgtaagtgactttttatttatttgtatttttgactgcattaagaggtctctagttttttatctcttgtttcccaaaacctaataagtaactaatgcacagagcacattgatttgtatttattctatttttagacataatttattagcatgcatgagcaaattaagaaaaacaacaacaaatgaatgcatatatatgtatatgtatgtgtgtatatatacacatatatatatatattttttttcttttcttaccagaaggttttaatccaaataaggagaagatatgcttagaactgaggtagagttttcatccattctgtcctgtaagtattttgcatattctggagacgcaggaagagatccatctacatatcccaaagctgaattatggtagacaaagctcttccacttttagtgcatcaatttcttatttgtgtaataagaaaattgggaaaacgatcttcaatatgcttaccaagctgtgattccaaatattacgtaaatacacttgcaaaggaggatgtttttagtagcaatttgtactgatggtatggggccaagagatatatcttagagggagggctgagggtttgaagtccaactcctaagccagtgccagaagagccaaggacaggtacggctgtcatcacttagacctcaccctgtggagccacaccctagggttggccaatctactcccaggagcagggagggcaggagccagggctgggcataaaagtcagggcagagccatctattgcttacatttgcttctgacacaactgtgttcactagcaacctcaaacagacaccatggtgcacctgactcctgaggagaagtctgccgttactgccctgtggggcaaggtgaacgtggatgaagttggtggtgaggccctgggcaggttggtatcaaggttacaagacaggtttaaggagaccaatagaaactgggcatgtggagacagagaagactcttgggtttctgataggcactgactctctctgcctattggtctattttcccacccttaggctgctggtggtctacccttggacccagaggttctttgagtcctttggggatctgtccactcctgatgctgttatgggcaaccctaaggtgaaggctcatggcaagaaagtgctcggtgcctttagtgatggcctggctcacctggacaacctcaagggcacctttgccacactgagtgagctgcactgtgacaagctgcacgtggatcctgagaacttcagggtgagtctatgggacccttgatgttttctttccccttcttttctatggttaagttcatgtcataggaaggggagaagtaacagggtacagtttagaatgggaaacagacgaatgattgcatcagtgtggaagtctcaggatcgttttagtttcttttatttgctgttcataacaattgttttcttttgtttaattcttgctttctttttttttcttctccgcaatttttactattatacttaatgccttaacattgtgtataacaaaaggaaatatctctgagatacattaagtaacttaaaaaaaaactttacacagtctgcctagtacattactatttggaatatatgtgtgcttatttgcatattcataatctccctactttattttcttttatttttaattgatacataatcattatacatatttatgggttaaagtgtaatgttttaatatgtgtacacatattgaccaaatcagggtaattttgcatttgtaattttaaaaaatgctttcttcttttaatatacttttttgtttatcttatttctaatactttccctaatctctttctttcagggcaataatgatacaatgtatcatgcctctttgcaccattctaaagaataacagtgataatttctgggttaaggcaatagcaatatttctgcatataaatatttctgcatataaattgtaactgatgtaagaggtttcatattgctaatagcagctacaatccagctaccattctgcttttattttatggttgggataaggctggattattctgagtccaagctaggcccttttgctaatcatgttcatacctcttatcttcctcccacagctcctgggcaacgtgctggtctgtgtgctggcccatcactttggcaaagaattcaccccaccagtgcaggctgcctatcagaaagtggtggctggtgtggctaatgccctggcccacaagtatcactaagctcgctttcttgctgtccaatttctattaaaggttcctttgttccctaagtccaactactaaactgggggatattatgaagggccttgagcatctggattctgcctaataaaaaacatttattttcattgcaatgatgtatttaaattatttctgaatattttactaaaaagggaatgtgggaggtcagtgcatttaaaacataaagaaatgaagagctagttcaaaccttgggaaaatacactatatcttaaactccatgaaagaaggtgaggctgcaaacagctaatgcacattggcaacagccctgatgcctatgccttattcatccctcagaaaaggattcaagtagaggcttgatttggaggttaaagttttgctatgctgtattttacattacttattgttttagctgtcctcatgaatgtcttttcactacccatttgcttatcctgcatctctcagccttgactccactcagttctcttgcttagagataccacctttcccctgaagtgttccttccatgttttacggcgagatggtttctcctcgcctggccactcagccttagttgtctctgttgtcttatagaggtctacttgaagaaggaaaaacagggggcatggtttgactgtcctgtgagcccttcttccctgcctcccccactcacagtgacccggaatctgcagtgctagtctcccggaactatcactctttcacagtctgctttggaaggactgggcttagtatgaaaagttaggactgagaagaatttgaaagggggctttttgtagcttgatattcactactgtcttattaccctatcataggcccaccccaaatggaagtcccattcttcctcaggatgtttaagattagcattcaggaagagatcagaggtctgctggctcccttatcatgtcccttatggtgcttctggctctgcagttattagcatagtgttaccatcaaccaccttaacttcatttttcttattcaatacctaggtaggtagatgctagattctggaaataaaatatgagtctcaagtggtccttgtcctctctcccagtcaaattctgaatctagttggcaagattctgaaatcaaggcatataatcagtaataagtgatgatagaagggtatatagaagaattttattatatgagagggtgaaacctaaaatgaaatgaaatcagacccttgtcttacaccataaacaaaaataaatttgaatgggttaaagaattaaactaagacctaaaaccataaaaatttttaaagaaatcaaaagaagaaaattctaatattcatgttgcagccgttttttgaatttgatatgagaagcaaaggcaacaaaaggaaaaataaagaagtgaggctacatcaaactaaaaaatttccacacaaaaaagaaaacaatgaacaaatgaaaggtgaaccatgaaatggcatatttgcaaaccaaatatttcttaaatattttggttaatatccaaaatatataagaaacacagatgattcaataacaaacaaaaaattaaaaataggaaaataaaaaaattaaaaagaagaaaatcctgccatttatgcgagaattgatgaacctggaggatgtaaaactaagaaaaataagcctgacacaaaaagacaaatactacacaaccttgctcatatgtgaaacataaaaaagtcactctcatggaaacagacagtagaggtatggtttccaggggttgggggtgggagaatcaggaaactattactcaaagggtataaaatttcagttatgtgggatgaataaattctagatatctaatgtacagcatcgtgactgtagttaattgtactgtaagtatatttaaaatttgcaaagagagtagatttttttgtttttttagatggagttttgctcttgttgtccaggctggagtgcaatggcaagatcttggctcactgcaacctccgcctcctgggttcaagcaaatctcctgcctcagcctcccgagtagctgggattacaggcatgcgacaccatgcccagctaattttgtatttttagtagagacggggtttctccatgttggtcaggctgatccgcctcctcggccaccaaagggctgggattacaggcgtgaccaccgggcctggccgagagtagatcttaaaagcatttaccacaagaaaaaggtaactatgtgagataatgggtatgttaattagcttgattgtggtaatcatttcacaaggtatacatatattaaaacatcatgttgtacaccttaaatatatacaatttttatttgtgaatgatacctcaataaagttgaagaataataaaaaagaatagacatcacatgaattaaaaaactaaaaaataaaaaaatgcatcttgatgattagaattgcattcttgatttttcagatacaaatatccatttgactg

SEQ ID NO: 43 - DNA, 60 bp, Artificial Sequence
  synthetic polynucleotide
  misc_feature (1)..(2): optional phosphorothioate internucleoside linkage
  misc_feature (2)..(3): optional phosphorothioate internucleoside linkage
  misc_feature (3)..(4): optional phosphorothioate internucleoside linkage
  misc_feature (57)..(58): optional phosphorothioate internucleoside linkage
  misc_feature (58)..(59): optional phosphorothioate internucleoside linkage
  misc_feature (59)..(60): optional phosphorothioate internucleoside linkage
aaagaataacagtgataatttctgggttaaggcaatagcaatatctctgcatataaatat

SEQ ID NO: 44 - DNA, 51 bp, Artificial Sequence
  synthetic polynucleotide
  misc_feature (1)..(2): optional phosphorothioate internucleoside linkage
  misc_feature (2)..(3): optional phosphorothioate internucleoside linkage
  misc_feature (3)..(4): optional phosphorothioate internucleoside linkage
  misc_feature (48)..(49): optional phosphorothioate internucleoside linkage
  misc_feature (49)..(50): optional phosphorothioate internucleoside linkage
  misc_feature (50)..(51): optional phosphorothioate internucleoside linkage
gttcagcgtgtccggcgagggcgaggtgagtctatgggacccttgatgttt

SEQ ID NO: 45 - DNA, 51 bp, Artificial Sequence
  synthetic polynucleotide
  misc_feature (1)..(2): optional phosphorothioate internucleoside linkage
  misc_feature (2)..(3): optional phosphorothioate internucleoside linkage
  misc_feature (3)..(4): optional phosphorothioate internucleoside linkage
  misc_feature (48)..(49): optional phosphorothioate internucleoside linkage
  misc_feature (49)..(50): optional phosphorothioate internucleoside linkage
  misc_feature (50)..(51): optional phosphorothioate internucleoside linkage
aaacatcaagggtcccatagactcacctcgccctcgccggacacgctgaac

SEQ ID NO: 46 - DNA, 70 bp, Artificial Sequence
  synthetic polynucleotide
  misc_feature (1)..(2): optional phosphorothioate internucleoside linkage
  misc_feature (2)..(3): optional phosphorothioate internucleoside linkage
  misc_feature (3)..(4): optional phosphorothioate internucleoside linkage
  misc_feature (67)..(68): optional phosphorothioate internucleoside linkage
  misc_feature (68)..(69): optional phosphorothioate internucleoside linkage
  misc_feature (69)..(70): optional phosphorothioate internucleoside linkage
cttgccccacagggcagtaacggcagatttttcttccggcgttaaatgcaccatggtgtctgtttgaggt

SEQ ID NO: 47 - DNA, 51 bp, Artificial Sequence
  synthetic polynucleotide
  misc_feature (1)..(2): optional phosphorothioate internucleoside linkage
  misc_feature (2)..(3): optional phosphorothioate internucleoside linkage
  misc_feature (3)..(4): optional phosphorothioate internucleoside linkage
  misc_feature (48)..(49): optional phosphorothioate internucleoside linkage
  misc_feature (49)..(50): optional phosphorothioate internucleoside linkage
  misc_feature (50)..(51): optional phosphorothioate internucleoside linkage
acagacaccatggtgcacctgactcctgaggagaagtctgccgttactgcc

SEQ ID NO: 48 - DNA, 65 bp, Artificial Sequence
  synthetic polynucleotide
  misc_feature (1)..(2): optional phosphorothioate internucleoside linkage
  misc_feature (2)..(3): optional phosphorothioate internucleoside linkage
  misc_feature (3)..(4): optional phosphorothioate internucleoside linkage
  misc_feature (62)..(63): optional phosphorothioate internucleoside linkage
  misc_feature (63)..(64): optional phosphorothioate internucleoside linkage
  misc_feature (64)..(65): optional phosphorothioate internucleoside linkage
ttgccccacagggcagtaacggcagacttctcctcaggagtcaggtgcaccatggtgtctgtttg

SEQ ID NO: 49 - DNA, 61 bp, Artificial Sequence
  synthetic polynucleotide
  misc_feature (1)..(2): optional phosphorothioate internucleoside linkage
  misc_feature (2)..(3): optional phosphorothioate internucleoside linkage
  misc_feature (3)..(4): optional phosphorothioate internucleoside linkage
  misc_feature (58)..(59): optional phosphorothioate internucleoside linkage
  misc_feature (59)..(60): optional phosphorothioate internucleoside linkage
  misc_feature (60)..(61): optional phosphorothioate internucleoside linkage
ttctgtatctatattcatcataggaaacaccaaagataatgttctccttaatggtgccagg

SEQ ID NO: 50 - DNA, 61 bp, Artificial Sequence
  synthetic polynucleotide
  misc_feature (1)..(2): optional phosphorothioate internucleoside linkage
  misc_feature (2)..(3): optional phosphorothioate internucleoside linkage
  misc_feature (3)..(4): optional phosphorothioate internucleoside linkage
  misc_feature (58)..(59): optional phosphorothioate internucleoside linkage
  misc_feature (59)..(60): optional phosphorothioate internucleoside linkage
  misc_feature (60)..(61): optional phosphorothioate internucleoside linkage
tcttgggattcaataaccttgcagacagtggaggaaggcctttggcgtgataccacaggtg

SEQ ID NO: 51 - DNA, 63 bp, Artificial Sequence
  synthetic polynucleotide
  misc_feature (1)..(2): optional phosphorothioate internucleoside linkage
  misc_feature (2)..(3): optional phosphorothioate internucleoside linkage
  misc_feature (3)..(4): optional phosphorothioate internucleoside linkage
  misc_feature (60)..(61): optional phosphorothioate internucleoside linkage
  misc_feature (61)..(62): optional phosphorothioate internucleoside linkage
  misc_feature (62)..(63): optional phosphorothioate internucleoside linkage
tccaagtttgcagagaaagataatatagtccttggagaaggaggaatcaccctgagtggaggt

SEQ ID NO: 52 - DNA, 64 bp, Artificial Sequence
  synthetic polynucleotide
  misc_feature (1)..(2): optional phosphorothioate internucleoside linkage
  misc_feature (2)..(3): optional phosphorothioate internucleoside linkage
  misc_feature (3)..(4): optional phosphorothioate internucleoside linkage
  misc_feature (61)..(62): optional phosphorothioate internucleoside linkage
  misc_feature (62)..(63): optional phosphorothioate internucleoside linkage
  misc_feature (63)..(64): optional phosphorothioate internucleoside linkage
aggacggtcccggcctgcgacacttccgcccataattgttcttcatctgcggggcggggggggg

SEQ ID NO: 53 - DNA, 67 bp, Artificial Sequence
  synthetic polynucleotide
  misc_feature (1)..(2): optional phosphorothioate internucleoside linkage
  misc_feature (2)..(3): optional phosphorothioate internucleoside linkage
  misc_feature (3)..(4): optional phosphorothioate internucleoside linkage
  misc_feature (64)..(65): optional phosphorothioate internucleoside linkage
  misc_feature (65)..(66): optional phosphorothioate internucleoside linkage
  misc_feature (66)..(67): optional phosphorothioate internucleoside linkage
gggacggcgcccacataggccaaattcaattgctgatcccagcttaagacgtactggtcagcctggc